European Patent Application EP 4 122 955 A1, published January 25, 2023. Title: SOLUBLE FIBROBLAST GROWTH FACTOR RECEPTOR 3 (SFGFR3) POLYPEPTIDES AND USES THEREOF. Applicant: Pfizer Inc. et al. The sequence listing filed with the application follows.

SEQUENCE LISTING (39 sequences)

SEQ ID NO: 1 - protein, 301 aa, Artificial Sequence
  Synthetic construct
ESLGTEQRVVGRAAEVPGPEPGQQEQLVFGSGDAVELSCPPPGGGPMGPTVWVKDGTGLVPSERVLVGPQRLQVLNASHEDSGAYSCRQRLTQRVLCHFSVRVTDAPSSGDDEDGEDEAEDTGVDTGAPYWTRPERMDKKLLAVPAANTVRFRCPAAGNPTPSISWLKNGREFRGEHRIGGIKLRHQQWSLVMESVVPSDRGNYTCVVENKFGSIRQTYTLDVLERSPHRPILQAGLPANQTAVLGSDVEFHCKVYSDAQPHIQWLKHVEVNGSKVGPDGTPYVTVLKVSLESNASMSSNT

SEQ ID NO: 2 - protein, 301 aa, Artificial Sequence
  Synthetic construct
ESLGTEQRVVGRAAEVPGPEPGQQEQLVFGSGDAVELSCPPPGGGPMGPTVWVKDGTGLVPSERVLVGPQRLQVLNASHEDSGAYSCRQRLTQRVLCHFSVRVTDAPSSGDDEDGEDEAEDTGVDTGAPYWTRPERMDKKLLAVPAANTVRFRCPAAGNPTPSISWLKNGREFRGEHRIGGIKLRHQQWSLVMESVVPSDRGNYTCVVENKFGSIRQTYTLDVLERSPHRPILQAGLPANQTAVLGSDVEFHSKVYSDAQPHIQWLKHVEVNGSKVGPDGTPYVTVLKVSLESNASMSSNT

SEQ ID NO: 3 - protein, 47 aa, Artificial Sequence
  Synthetic construct
TAGANTTDKELEVLSLNVTFEDAGEYTCLAGNSIGFSHHSAWLVVLP

SEQ ID NO: 4 - protein, 348 aa, Artificial Sequence
  Synthetic construct
ESLGTEQRVVGRAAEVPGPEPGQQEQLVFGSGDAVELSCPPPGGGPMGPTVWVKDGTGLVPSERVLVGPQRLQVLNASHEDSGAYSCRQRLTQRVLCHFSVRVTDAPSSGDDEDGEDEAEDTGVDTGAPYWTRPERMDKKLLAVPAANTVRFRCPAAGNPTPSISWLKNGREFRGEHRIGGIKLRHQQWSLVMESVVPSDRGNYTCVVENKFGSIRQTYTLDVLERSPHRPILQAGLPANQTAVLGSDVEFHCKVYSDAQPHIQWLKHVEVNGSKVGPDGTPYVTVLKTAGANTTDKELEVLSLNVTFEDAGEYTCLAGNSIGFSHHSAWLVVLPVSLESNASMSSNT

SEQ ID NO: 5 - protein, 784 aa, Homo sapiens
ESLGTEQRVVGRAAEVPGPEPGQQEQLVFGSGDAVELSCPPPGGGPMGPTVWVKDGTGLVPSERVLVGPQRLQVLNASHEDSGAYSCRQRLTQRVLCHFSVRVTDAPSSGDDEDGEDEAEDTGVDTGAPYWTRPERMDKKLLAVPAANTVRFRCPAAGNPTPSISWLKNGREFRGEHRIGGIKLRHQQWSLVMESVVPSDRGNYTCVVENKFGSIRQTYTLDVLERSPHRPILQAGLPANQTAVLGSDVEFHCKVYSDAQPHIQWLKHVEVNGSKVGPDGTPYVTVLKTAGANTTDKELEVLSLHNVTFEDAGEYTCLAGNSIGFSHHSAWLVVLPAEEELVEADEAGSVYAGILSYGVGFFLFILVVAAVTLCRLRSPPKKGLGSPTVHKISRFPLKRQVSLESNASMSSNTPLVRIARLSSGEGPTLANVSELELPADPKWELSRARLTLGKPLGEGCFGQVVMAEAIGIDKDRAAKPVTVAVKMLKDDATDKDLSDLVSEMEMMKMIGKHKNIINLLGACTQGGPLYVLVEYAAKGNLREFLRARRPPGLDYSFDTCKPPEEQLTFKDLVSCAYQVARGMEYLASQKCIHRDLAARNVLVTEDNVMKIADFGLARDVHNLDYYKKTTNGRLPVKWMAPEALFDRVYTHQSDVWSFGVLLWEIFTLGGSPYPGIPVEELFKLLKEGHRMDKPANCTHDLYMIMRECWHAAPSQRPTFKQLVEDLDRVLTVTSTDEYLDLSAPFEQYSPGGQDTPSSSSSGDDSVFAHDLLPPAPPSSGGSRT

SEQ ID NO: 6 - protein, 22 aa, Artificial Sequence
  Synthetic construct
MGAPACALALCVAVAIVAGASS

SEQ ID NO: 7 - protein, 672 aa, Homo sapiens
ESLGTEQRVVGRAAEVPGPEPGQQEQLVFGSGDAVELSCPPPGGGPMGPTVWVKDGTGLVPSERVLVGPQRLQVLNASHEDSGAYSCRQRLTQRVLCHFSVRVTDAPSSGDDEDGEDEAEDTGVDTGAPYWTRPERMDKKLLAVPAANTVRFRCPAAGNPTPSISWLKNGREFRGEHRIGGIKLRHQQWSLVMESVVPSDRGNYTCVVENKFGSIRQTYTLDVLERSPHRPILQAGLPANQTAVLGSDVEFHCKVYSDAQPHIQWLKHVEVNGSKVGPDGTPYVTVLKVSLESNASMSSNTPLVRIARLSSGEGPTLANVSELELPADPKWELSRARLTLGKPLGEGCFGQVVMAEAIGIDKDRAAKPVTVAVKMLKDDATDKDLSDLVSEMEMMKMIGKHKNIINLLGACTQGGPLYVLVEYAAKGNLREFLRARRPPGLDYSFDTCKPPEEQLTFKDLVSCAYQVARGMEYLASQKCIHRDLAARNVLVTEDNVMKIADFGLARDVHNLDYYKKTTNGRLPVKWMAPEALFDRVYTHQSDVWSFGVLLWEIFTLGGSPYPGIPVEELFKLLKEGHRMDKPANCTHDLYMIMRECWHAAPSQRPTFKQLVEDLDRVLTVTSTDEYLDLSAPFEQYSPGGQDTPSSSSSGDDSVFAHDLLPPAPPSSGGSRT

SEQ ID NO: 8 - protein, 672 aa, Artificial Sequence
  Synthetic construct
ESLGTEQRVVGRAAEVPGPEPGQQEQLVFGSGDAVELSCPPPGGGPMGPTVWVKDGTGLVPSERVLVGPQRLQVLNASHEDSGAYSCRQRLTQRVLCHFSVRVTDAPSSGDDEDGEDEAEDTGVDTGAPYWTRPERMDKKLLAVPAANTVRFRCPAAGNPTPSISWLKNGREFRGEHRIGGIKLRHQQWSLVMESVVPSDRGNYTCVVENKFGSIRQTYTLDVLERSPHRPILQAGLPANQTAVLGSDVEFHSKVYSDAQPHIQWLKHVEVNGSKVGPDGTPYVTVLKVSLESNASMSSNTPLVRIARLSSGEGPTLANVSELELPADPKWELSRARLTLGKPLGEGCFGQVVMAEAIGIDKDRAAKPVTVAVKMLKDDATDKDLSDLVSEMEMMKMIGKHKNIINLLGACTQGGPLYVLVEYAAKGNLREFLRARRPPGLDYSFDTCKPPEEQLTFKDLVSCAYQVARGMEYLASQKCIHRDLAARNVLVTEDNVMKIADFGLARDVHNLDYYKKTTNGRLPVKWMAPEALFDRVYTHQSDVWSFGVLLWEIFTLGGSPYPGIPVEELFKLLKEGHRMDKPANCTHDLYMIMRECWHAAPSQRPTFKQLVEDLDRVLTVTSTDEYLDLSAPFEQYSPGGQDTPSSSSSGDDSVFAHDLLPPAPPSSGGSRT

SEQ ID NO: 9 - protein, 720 aa, Artificial Sequence
  Synthetic construct
ESLGTEQRVVGRAAEVPGPEPGQQEQLVFGSGDAVELSCPPPGGGPMGPTVWVKDGTGLVPSERVLVGPQRLQVLNASHEDSGAYSCRQRLTQRVLCHFSVRVTDAPSSGDDEDGEDEAEDTGVDTGAPYWTRPERMDKKLLAVPAANTVRFRCPAAGNPTPSISWLKNGREFRGEHRIGGIKLRHQQWSLVMESVVPSDRGNYTCVVENKFGSIRQTYTLDVLERSPHRPILQAGLPANQTAVLGSDVEFHCKVYSDAQPHIQWLKHVEVNGSKVGPDGTPYVTVLKTAGANTTDKELEVLSLHNVTFEDAGEYTCLAGNSIGFSHHSAWLVVLPVSLESNASMSSNTPLVRIARLSSGEGPTLANVSELELPADPKWELSRARLTLGKPLGEGCFGQVVMAEAIGIDKDRAAKPVTVAVKMLKDDATDKDLSDLVSEMEMMKMIGKHKNIINLLGACTQGGPLYVLVEYAAKGNLREFLRARRPPGLDYSFDTCKPPEEQLTFKDLVSCAYQVARGMEYLASQKCIHRDLAARNVLVTEDNVMKIADFGLARDVHNLDYYKKTTNGRLPVKWMAPEALFDRVYTHQSDVWSFGVLLWEIFTLGGSPYPGIPVEELFKLLKEGHRMDKPANCTHDLYMIMRECWHAAPSQRPTFKQLVEDLDRVLTVTSTDEYLDLSAPFEQYSPGGQDTPSSSSSGDDSVFAHDLLPPAPPSSGGSRT

SEQ ID NO: 10 - protein, 512 aa, Artificial Sequence
  Synthetic construct
ESLGTEQRVVGRAAEVPGPEPGQQEQLVFGSGDAVELSCPPPGGGPMGPTVWVKDGTGLVPSERVLVGPQRLQVLNASHEDSGAYSCRQRLTQRVLCHFSVRVTDAPSSGDDEDGEDEAEDTGVDTGAPYWTRPERMDKKLLAVPAANTVRFRCPAAGNPTPSISWLKNGREFRGEHRIGGIKLRHQQWSLVMESVVPSDRGNYTCVVENKFGSIRQTYTLDVLERSPHRPILQAGLPANQTAVLGSDVEFHCKVYSDAQPHIQWLKHVEVNGSKVGPDGTPYVTVLKVSLESNASMSSNTSGSGSGSGSGSGSGSVVFPYFPRLGRYNLNFHEAQQACLDQDAVIASFDQLYDAWRGGLDWCNAGWLSDGSVQYPITKPREPCGGQNTVPGVRNYGFWDKDKSRYDVFCFTSNFNGRFYYLIHPTKLTYDEAVQACLNDGAQIAKVGQIFAAWKILGYDRCDAGWLADGSVRYPISRPRRRCSPTEAAVRFVGFPDKKHKLYGVYCFRAYN

SEQ ID NO: 11 - protein, 512 aa, Artificial Sequence
  Synthetic construct
ESLGTEQRVVGRAAEVPGPEPGQQEQLVFGSGDAVELSCPPPGGGPMGPTVWVKDGTGLVPSERVLVGPQRLQVLNASHEDSGAYSCRQRLTQRVLCHFSVRVTDAPSSGDDEDGEDEAEDTGVDTGAPYWTRPERMDKKLLAVPAANTVRFRCPAAGNPTPSISWLKNGREFRGEHRIGGIKLRHQQWSLVMESVVPSDRGNYTCVVENKFGSIRQTYTLDVLERSPHRPILQAGLPANQTAVLGSDVEFHSKVYSDAQPHIQWLKHVEVNGSKVGPDGTPYVTVLKVSLESNASMSSNTSGSGSGSGSGSGSGSVVFPYFPRLGRYNLNFHEAQQACLDQDAVIASFDQLYDAWRGGLDWCNAGWLSDGSVQYPITKPREPCGGQNTVPGVRNYGFWDKDKSRYDVFCFTSNFNGRFYYLIHPTKLTYDEAVQACLNDGAQIAKVGQIFAAWKILGYDRCDAGWLADGSVRYPISRPRRRCSPTEAAVRFVGFPDKKHKLYGVYCFRAYN

SEQ ID NO: 12 - protein, 560 aa, Artificial Sequence
  Synthetic construct
ESLGTEQRVVGRAAEVPGPEPGQQEQLVFGSGDAVELSCPPPGGGPMGPTVWVKDGTGLVPSERVLVGPQRLQVLNASHEDSGAYSCRQRLTQRVLCHFSVRVTDAPSSGDDEDGEDEAEDTGVDTGAPYWTRPERMDKKLLAVPAANTVRFRCPAAGNPTPSISWLKNGREFRGEHRIGGIKLRHQQWSLVMESVVPSDRGNYTCVVENKFGSIRQTYTLDVLERSPHRPILQAGLPANQTAVLGSDVEFHCKVYSDAQPHIQWLKHVEVNGSKVGPDGTPYVTVLKTAGANTTDKELEVLSLHNVTFEDAGEYTCLAGNSIGFSHHSAWLVVLPVSLESNASMSSNTSGSGSGSGSGSGSGSVVFPYFPRLGRYNLNFHEAQQACLDQDAVIASFDQLYDAWRGGLDWCNAGWLSDGSVQYPITKPREPCGGQNTVPGVRNYGFWDKDKSRYDVFCFTSNFNGRFYYLIHPTKLTYDEAVQACLNDGAQIAKVGQIFAAWKILGYDRCDAGWLADGSVRYPISRPRRRCSPTEAAVRFVGFPDKKHKLYGVYCFRAYN

SEQ ID NO: 13 - protein, 155 aa, Homo sapiens
MAEGEITTFTALTEKFNLPPGNYKKPKLLYCSNGGHFLRILPDGTVDGTRDRSDQHIQLQLSAESVGEVYIKSTETGQYLAMDTDGLLYGSQTPNEECLFLERLEENHYNTYISKKHAEKNWFVGLKKNGSCKRGPRTHYGQKAILFLPLPVSSD

SEQ ID NO: 14 - protein, 288 aa, Homo sapiens
MVGVGGGDVEDVTPRPGGCQISGRGARGCNGIPGAAAWEAALPRRRPRRHPSVNPRSRAAGSPRTRGRRTEERPSGSRLGDRGRGRALPGGRLGGRGRGRAPERVGGRGRGRGTAAPRAAPAARGSRPGPAGTMAAGSITTLPALPEDGGSGAFPPGHFKDPKRLYCKNGGFFLRIHPDGRVDGVREKSDPHIKLQLQAEERGVVSIKGVCANRYLAMKEDGRLLASKCVTDECFFFERLESNNYNTYRSRKYTSWYVALKRTGQYKLGSKTGPGQKAILFLPMSAKS

SEQ ID NO: 15 - protein, 208 aa, Homo sapiens
MAPLGEVGNYFGVQDAVPFGNVPVLPVDSPVLLSDHLGQSEAGGLPRGPAVTDLDHLKGILRRRQLYCRTGFHLEIFPNGTIQGTRKDHSRFGILEFISIAVGLVSIRGVDSGLYLGMNEKGELYGSEKLTQECVFREQFEENWYNTYSSNLYKHVDTGRRYYVALNKDGTPREGTRTKRHQKFTHFLPRPVDPDKVPELYKDILSQS

SEQ ID NO: 16 - protein, 207 aa, Homo sapiens
MYSAPSACTCLCLHFLLLCFQVQVLVAEENVDFRIHVENQTRARDDVSRKQLRLYQLYSRTSGKHIQVLGRRISARGEDGDKYAQLLVETDTFGSQVRIKGKETEFYLCMNRKGKLVGKPDGTSKECVFIEKVLENNYTALMSAKYSGWYVGFTKKGRPRKGPKTRENQQDVHFMKRYPKGQPELQKPFKYTTVTKRSRRIRPTHPA

SEQ ID NO: 17 - protein, 323 aa, Artificial Sequence
  Synthetic construct
MGAPACALALCVAVAIVAGASSESLGTEQRVVGRAAEVPGPEPGQQEQLVFGSGDAVELSCPPPGGGPMGPTVWVKDGTGLVPSERVLVGPQRLQVLNASHEDSGAYSCRQRLTQRVLCHFSVRVTDAPSSGDDEDGEDEAEDTGVDTGAPYWTRPERMDKKLLAVPAANTVRFRCPAAGNPTPSISWLKNGREFRGEHRIGGIKLRHQQWSLVMESVVPSDRGNYTCVVENKFGSIRQTYTLDVLERSPHRPILQAGLPANQTAVLGSDVEFHCKVYSDAQPHIQWLKHVEVNGSKVGPDGTPYVTVLKVSLESNASMSSNT

SEQ ID NO: 18 - protein, 323 aa, Artificial Sequence; identical to SEQ ID NO: 17
  Synthetic construct

SEQ ID NO: 19 - protein, 323 aa, Artificial Sequence
  Synthetic construct
MGAPACALALCVAVAIVAGASSESLGTEQRVVGRAAEVPGPEPGQQEQLVFGSGDAVELSCPPPGGGPMGPTVWVKDGTGLVPSERVLVGPQRLQVLNASHEDSGAYSCRQRLTQRVLCHFSVRVTDAPSSGDDEDGEDEAEDTGVDTGAPYWTRPERMDKKLLAVPAANTVRFRCPAAGNPTPSISWLKNGREFRGEHRIGGIKLRHQQWSLVMESVVPSDRGNYTCVVENKFGSIRQTYTLDVLERSPHRPILQAGLPANQTAVLGSDVEFHSKVYSDAQPHIQWLKHVEVNGSKVGPDGTPYVTVLKVSLESNASMSSNT

SEQ ID NO: 20 - DNA, 987 bp, Artificial Sequence
  Synthetic construct
atgggagtgaaggtgctgttcgccctgatctgtatcgccgtggccgaggccgagtctctgggcacagaacagagagtcgtgggcagagccgccgaagtgcctggacctgaacctggccagcaggaacagctggtgtttggcagcggcgacgccgtggaactgagctgtcctccacctggcggaggccctatgggacctaccgtgtgggtcaaggatggcaccggactggtgcctagcgagagggtgctcgtgggacctcagagactgcaggtgctgaacgccagccacgaggatagcggcgcctacagctgcagacagagactgacacagcgggtgctgtgccacttctccgtcagagtgaccgacgcccctagctccggcgacgatgaggatggcgaagatgaggccgaggacaccggcgtggacacaggcgctccatactggaccagacccgagcggatggacaagaaactgctggccgtgcctgccgccaacaccgtgcggtttagatgtcctgccgccggaaaccccacccccagcatcagctggctgaagaacggcagagagttccggggcgagcacagaatcggcggcatcaagctgagacaccagcagtggtccctcgtgatggaaagcgtggtgcccagcgaccggggcaactacacctgtgtggtggaaaacaagttcggcagcatccggcagacctacaccctggacgtgctggaaagaagcccccacagacccatcctgcaggccggactgcctgccaatcagacagccgtgctgggcagcgacgtggaatttcacagcaaggtgtacagcgacgcccagccccacatccagtggctgaaacacgtggaagtgaacggcagcaaagtgggccccgacggcaccccttatgtgaccgtgctgaaggtgtccctggaaagcaacgccagcatgagcagcaacaccgactacaaggacgacgacgacaagtgaaagctt

SEQ ID NO: 21 - DNA, 1131 bp, Artificial Sequence
  Synthetic construct
atgggagtgaaggtgctgttcgccctgatctgtatcgccgtggccgaggccgagtctctgggcacagaacagagagtcgtgggcagagccgccgaagtgcctggacctgaacctggccagcaggaacagctggtgtttggcagcggcgacgccgtggaactgagctgtcctccacctggcggaggccctatgggacctaccgtgtgggtcaaggatggcaccggactggtgcctagcgagagggtgctcgtgggacctcagagactgcaggtgctgaacgccagccacgaggatagcggcgcctacagctgcagacagagactgacacagcgggtgctgtgccacttctccgtcagagtgaccgacgcccctagctccggcgacgatgaggatggcgaagatgaggccgaggacaccggcgtggacacaggcgctccatactggaccagacccgagcggatggacaagaaactgctggccgtgcctgccgccaacaccgtgcggtttagatgtcctgccgccggaaaccccacccccagcatcagctggctgaagaacggcagagagttccggggcgagcacagaatcggcggcatcaagctgagacaccagcagtggtccctcgtgatggaaagcgtggtgcccagcgaccggggcaactacacctgtgtggtggaaaacaagttcggcagcatccggcagacctacaccctggacgtgctggaaagaagcccccacagacccatcctgcaggccggactgcctgccaatcagacagccgtgctgggcagcgacgtggaatttcactgcaaggtgtacagcgacgcccagccccacatccagtggctgaaacacgtggaagtgaacggcagcaaagtgggccccgacggcaccccttatgtgaccgtgctgaaaaccgctggcgccaataccaccgacaaagaactggaagtgctgagcctgcacaacgtgaccttcgaggatgccggcgagtacacctgtctggccggcaacagcatcggcttcagccaccattctgcctggctggtggtgctgcccgtgtccctggaaagcaacgccagcatgagcagcaacaccgactacaaggacgacgacgacaagtgaaagctt

SEQ ID NO: 22 - DNA, 2019 bp, Artificial Sequence
  Synthetic construct
atggagtctctgggcacagagcagagagtcgtgggcagagccgctgaagtgcctggacctgagcctggccagcaggaacagctggtctttggctctggcgacgccgtggaactgagctgtcctccacctggcggaggccctatgggacctaccgtgtgggtcaaggatggcaccggactggtgcctagcgagagggtgctcgtgggacctcagagactgcaggtcctgaacgccagccacgaggatagcggcgcctacagctgcagacagagactgacccagcgggtgctgtgccacttcagcgtcagagtgaccgatgcccccagcagcggagatgacgaggatggcgaggatgaggccgaggatacaggcgtggacacaggcgccccttactggaccagacccgagcggatggacaagaaactgctggccgtgcctgccgccaacaccgtgcggtttagatgccctgccgccggaaaccccacccccagcatctcttggctgaagaacggcagagagttccggggcgagcaccggatcggcggcattaagctgagacaccagcagtggtccctggtcatggaaagcgtggtgcccagcgaccggggcaactacacctgtgtggtggaaaacaagttcggcagcatccggcagacctacaccctggacgtgctggaaagaagcccccacagacctatcctgcaggccggactgcctgccaatcagacagccgtgctgggcagcgacgtggaatttcacagcaaggtgtacagcgacgcccagccccacatccagtggctgaagcacgtggaagtgaacggcagcaaagtgggccccgacggcaccccttacgtgaccgtgctgaaagtgtccctggaaagcaacgccagcatgagcagcaacacccccctcgtgcggatcgccagactgtctagcggagagggccctaccctggccaacgtgtccgaactggaactgcccgccgaccccaagtgggagctgagcagagctagactgaccctgggcaagcctctgggcgagggctgttttggacaggtggtcatggccgaggccatcggcatcgacaaggacagagccgccaagcctgtgaccgtggccgtgaagatgctgaaggacgacgccaccgacaaggacctgagcgacctggtgtccgagatggaaatgatgaagatgatcggcaagcacaagaacatcatcaacctgctgggcgcctgcacccagggcggacctctgtacgtgctggtggaatacgccgccaagggcaacctgagagagttcctgagagccagaaggccccctggcctggactacagcttcgatacctgcaagccccccgaagaacagctgaccttcaaggatctggtgtcctgcgcctatcaggtggccagaggcatggaatacctggccagccagaagtgcatccaccgggatctggccgccagaaacgtgctggtcaccgaggacaacgtgatgaagatcgccgacttcggcctggcccgggacgtgcacaacctggactactacaagaaaaccaccaacggccggctgcccgtgaagtggatggcccctgaggccctgttcgacagagtgtacacccaccagagcgacgtgtggtccttcggcgtgctgctgtgggagatctttaccctgggcggcagcccttaccccggcatccctgtggaagaactgttcaagctgctgaaagagggccacagaatggacaagcccgccaactgcacccacgacctgtacatgatcatgagagagtgctggcacgccgctcccagccagaggcctacctttaagcagctggtggaagatctggaccgggtgctgaccgtgaccagcaccgacgagtacctggatctgagcgcccccttcgagcagtactctcctggcggccaggatacccctagcagcagctctagcggcgacgacagcgtgttcgcccacgatctgctgcctccagcccctcctagctctggcggctctagaacc

SEQ ID NO: 23 - DNA, 1491 bp, Artificial Sequence
  Synthetic construct
atggagagcctgggcacagaacagagagtcgtgggcagagccgccgaagtgcctggacctgaacctggccagcaggaacagctggtctttggctctggcgacgccgtggaactgagctgtcctccacctggcggaggccctatgggacctaccgtgtgggtcaaggatggcaccggactggtgcctagcgagagggtgctcgtgggacctcagagactgcaggtcctgaacgccagccacgaggatagcggcgcctacagctgcagacagagactgacccagcgggtgctgtgccacttcagcgtcagagtgaccgatgcccccagcagcggagatgacgaggatggcgaggatgaggccgaggatacaggcgtggacacaggcgccccttactggaccagacccgagcggatggacaagaaactgctggccgtgcctgccgccaacaccgtgcggtttagatgccctgccgccggaaaccccacccccagcatctcttggctgaagaacggcagagagttccggggcgagcaccggatcggcggcattaagctgagacaccagcagtggtccctggtcatggaaagcgtggtgcccagcgaccggggcaactacacctgtgtggtggaaaacaagttcggcagcatccggcagacctacaccctggacgtgctggaaagaagcccccacagacctatcctgcaggccggactgcctgccaatcagacagccgtgctgggcagcgacgtggaatttcactgcaaggtgtacagcgacgcccagccccacatccagtggctgaagcacgtggaagtgaacggcagcaaagtgggccccgacggcaccccttacgtgaccgtgctgaaagtgtccctggaaagcaacgccagcatgagcagcaacaccagcggcagcggctctggcagcggatctggttctggctccggcagcgtggtgttcccctacttcccccggctgggccggtacaacctgaactttcatgaggcccagcaggcctgcctggaccaggatgccgtgatcgccagcttcgaccagctgtacgatgcttggagaggcggcctggactggtgcaatgccggctggctgtctgacggcagcgtgcagtaccccatcaccaagcccagagagccctgcggcggacagaataccgtgcccggcgtgcggaactacggcttctgggacaaggacaagagcagatacgacgtgttctgcttcaccagcaacttcaacggccggttctactacctgatccaccccaccaagctgacctacgacgaggccgtgcaggcctgtctgaacgatggcgcccagatcgccaaagtgggacagatcttcgccgcctggaagatcctgggctacgacagatgtgacgccggatggctggccgacggctccgtgcggtatcccatcagccggcctagaagaagatgcagccctaccgaggccgccgtcagattcgtgggcttcccc

SEQ ID NO: 24 - DNA, 1710 bp, Artificial Sequence
  Synthetic construct
atgggagcaccagcttgtgccctggctctgtgtgtggccgtggctattgtggctggcgcctctagcgagagcctgggcacagaacagagagtcgtgggcagagccgccgaagtgcctggacctgaacctggccagcaggaacagctggtctttggctctggcgacgccgtggaactgagctgtcctccacctggcggaggccctatgggacctaccgtgtgggtcaaggatggcaccggactggtgcctagcgagagggtgctcgtgggacctcagagactgcaggtcctgaacgccagccacgaggatagcggcgcctacagctgcagacagagactgacccagcgggtgctgtgccacttcagcgtcagagtgaccgatgcccccagcagcggagatgacgaggatggcgaggatgaggccgaggatacaggcgtggacacaggcgccccttactggaccagacccgagcggatggacaagaaactgctggccgtgcctgccgccaacaccgtgcggtttagatgccctgccgccggaaaccccacccccagcatctcttggctgaagaacggcagagagttccggggcgagcaccggatcggcggcattaagctgagacaccagcagtggtccctggtcatggaaagcgtggtgcccagcgaccggggcaactacacctgtgtggtggaaaacaagttcggcagcatccggcagacctacaccctggacgtgctggaaagaagcccccacagacctatcctgcaggccggactgcctgccaatcagacagccgtgctgggcagcgacgtggaatttcactgcaaggtgtacagcgacgcccagccccacatccagtggctgaagcacgtggaagtgaacggcagcaaagtgggccccgacggcaccccttacgtgaccgtgctgaaaaccgctggcgccaacaccaccgacaaagaactggaagtgctgagcctgcacaacgtgaccttcgaggacgccggcgagtacacctgtctggccggcaatagcatcggcttcagccaccactctgcctggctggtggtgctgccaggcggaggctctgtgtccctggaaagcaacgccagcatgagcagcaacaccagcggcagcggctctggcagcggatctggttctggctccggcagcgtggtgttcccctacttcccccggctgggccggtacaacctgaactttcatgaggcccagcaggcctgcctggaccaggatgccgtgatcgccagcttcgaccagctgtacgatgcttggagaggcggcctggactggtgcaatgccggctggctgtctgacggcagcgtgcagtaccccatcaccaagcccagagagccctgcggcggacagaataccgtgcccggcgtgcggaactacggcttctgggacaaggacaagagcagatacgacgtgttctgcttcaccagcaacttcaacggccggttctactacctgatccaccccaccaagctgacctacgacgaggccgtgcaggcctgtctgaacgatggcgcccagatcgccaaagtgggacagatcttcgccgcctggaagatcctgggctacgacagatgtgacgccggatggctggccgacggctccgtgcggtatcccatcagccggcctagaagaagatgcagccctaccgaggccgccgtcagattcgtgggcttcccc

SEQ ID NO: 25 - protein, 236 aa, Homo sapiens
GGGGAGGGGDKTHTCPPCPAPELLGGPSVFLFPPKPKDTLMISRTPEVTCVVVDVSHEDPEVKFNWYVDGVEVHNAKTKPREEQYNSTYRVVSVLTVLHQDWLNGKEYKCKVSNKALPAPIEKTISKAKGQPREPQVYTLPPSRDELTKNQVSLTCLVKGFYPSDIAVEWESNGQPENNYKTTPPVLDSDGSFFLYSKLTVDKSRWQQGNVFSCSVMHEALHNHYTQKSLSLSPGK

SEQ ID NO: 26 - protein, 236 aa, Artificial Sequence
  Synthetic construct
GGGGAGGGGDKTHTCPPCPAPELLGGPSVFLFPPKPKDTLMISRTPEVTCVVVDVSHEDPEVKFNWYVDGVEVHNAKTKPREEQYASTYRVVSVLTVLHQDWLNGKEYKCKVSNKALPAPIEKTISKAKGQPREPQVYTLPPSREEMTKNQVSLTCLVKGFYPSDIAVEWESNGQPENNYKTTPPVLDSDGSFFLYSKLTVDKSRWQQGNVFSCSVMHEALHNHYTQKSLSLSPGK

SEQ ID NO: 27 - protein, 585 aa, Homo sapiens [sequence omitted]

SEQ ID NO: 28 - protein, 9 aa, Artificial Sequence
  Synthetic construct
GGGGAGGGG

SEQ ID NO: 29 - protein, 15 aa, Artificial Sequence
  Synthetic construct
GGGGSGGGGSGGGGS

SEQ ID NO: 30 - protein, 24 aa, Artificial Sequence
  Synthetic construct
AGGTGGCCTTTGACACCTACCAGG

SEQ ID NO: 31 - protein, 24 aa, Artificial Sequence
  Synthetic construct
TCTGTTGTGTTTCCTCCCTGTTGG

SEQ ID NO: 32 - protein, 806 aa, Artificial Sequence
  Synthetic construct
MGAPACALALCVAVAIVAGASSESLGTEQRVVGRAAEVPGPEPGQQEQLVFGSGDAVELSCPPPGGGPMGPTVWVKDGTGLVPSERVLVGPQRLQVLNASHEDSGAYSCRQRLTQRVLCHFSVRVTDAPSSGDDEDGEDEAEDTGVDTGAPYWTRPERMDKKLLAVPAANTVRFRCPAAGNPTPSISWLKNGREFRGEHRIGGIKLRHQQWSLVMESVVPSDRGNYTCVVENKFGSIRQTYTLDVLERSPHRPILQAGLPANQTAVLGSDVEFHCKVYSDAQPHIQWLKHVEVNGSKVGPDGTPYVTVLKTAGANTTDKELEVLSLHNVTFEDAGEYTCLAGNSIGFSHHSAWLVVLPAEEELVEADEAGSVYAGILSYGVGFFLFILVVAAVTLCRLRSPPKKGLGSPTVHKISRFPLKRQVSLESNASMSSNTPLVRIARLSSGEGPTLANVSELELPADPKWELSRARLTLGKPLGEGCFGQVVMAEAIGIDKDRAAKPVTVAVKMLKDDATDKDLSDLVSEMEMMKMIGKHKNIINLLGACTQGGPLYVLVEYAAKGNLREFLRARRPPGLDYSFDTCKPPEEQLTFKDLVSCAYQVARGMEYLASQKCIHRDLAARNVLVTEDNVMKIADFGLARDVHNLDYYKKTTNGRLPVKWMAPEALFDRVYTHQSDVWSFGVLLWEIFTLGGSPYPGIPVEELFKLLKEGHRMDKPANCTHDLYMIMRECWHAAPSQRPTFKQLVEDLDRVLTVTSTDEYLDLSAPFEQYSPGGQDTPSSSSSGDDSVFAHDLLPPAPPSSGGSRT

SEQ ID NO: 33 - protein, 349 aa, Artificial Sequence
  Synthetic construct
ESLGTEQRVVGRAAEVPGPEPGQQEQLVFGSGDAVELSCPPPGGGPMGPTVWVKDGTGLVPSERVLVGPQRLQVLNASHEDSGAYSCRQRLTQRVLCHFSVRVTDAPSSGDDEDGEDEAEDTGVDTGAPYWTRPERMDKKLLAVPAANTVRFRCPAAGNPTPSISWLKNGREFRGEHRIGGIKLRHQQWSLVMESVVPSDRGNYTCVVENKFGSIRQTYTLDVLERSPHRPILQAGLPANQTAVLGSDVEFHCKVYSDAQPHIQWLKHVEVNGSKVGPDGTPYVTVLKTAGANTTDKELEVLSLHNVTFEDAGEYTCLAGNSIGFSHHSAWLVVLPVSLESNASMSSNT

SEQ ID NO: 34 - protein, 368 aa, Artificial Sequence [sequence omitted]

SEQ ID NO: 35 - protein, 19 aa, Artificial Sequence
  Synthetic construct
MMSFVSLLLVGILFHATQA

SEQ ID NO: 36 - DNA, 963 bp, Artificial Sequence
  Synthetic construct
atgatgtcctttgtctctctgctcctggttggcatcctattccatgccacccaggccgagtccttggggacggagcagcgcgtcgtggggcgagcggcagaagtcccgggcccagagcccggccagcaggagcagttggtcttcggcagcggggatgctgtggagctgagctgtcccccgcccgggggtggtcccatggggcccactgtctgggtcaaggatggcacagggctggtgccctcggagcgtgtcctggtggggccccagcggctgcaggtgctgaatgcctcccacgaggactccggggcctacagctgccggcagcggctcacgcagcgcgtactgtgccacttcagtgtgcgggtgacagacgctccatcctcgggagatgacgaagacggggaggacgaggctgaggacacaggtgtggacacaggggccccttactggacacggcccgagcggatggacaagaagctgctggccgtgccggccgccaacaccgtccgcttccgctgcccagccgctggcaaccccactccctccatctcctggctgaagaacggcagggagttccgcggcgagcaccgcattggaggcatcaagctgcggcatcagcagtggagcctggtcatggaaagcgtggtgccctcggaccgcggcaactacacctgcgtcgtggagaacaagtttggcagcatccggcagacgtacacgctggacgtgctggagcgctccccgcaccggcccatcctgcaggcggggctgccggccaaccagacggcggtgctgggcagcgacgtggagttccactccaaggtgtacagtgacgcacagccccacatccagtggctcaagcacgtggaggtgaatggcagcaaggtgggcccggacggcacaccctacgttaccgtgctcaaggtgtccctggagtccaacgcgtccatgagctccaacacatga

SEQ ID NO: 37 - DNA, 1107 bp, Artificial Sequence
  Synthetic construct
atgatgtcctttgtctctctgctcctggttggcatcctattccatgccacccaggccgagtccttggggacggagcagcgcgtcgtggggcgagcggcagaagtcccgggcccagagcccggccagcaggagcagttggtcttcggcagcggggatgctgtggagctgagctgtcccccgcccgggggtggtcccatggggcccactgtctgggtcaaggatggcacagggctggtgccctcggagcgtgtcctggtggggccccagcggctgcaggtgctgaatgcctcccacgaggactccggggcctacagctgccggcagcggctcacgcagcgcgtactgtgccacttcagtgtgcgggtgacagacgctccatcctcgggagatgacgaagacggggaggacgaggctgaggacacaggtgtggacacaggggccccttactggacacggcccgagcggatggacaagaagctgctggccgtgccggccgccaacaccgtccgcttccgctgcccagccgctggcaaccccactccctccatctcctggctgaagaacggcagggagttccgcggcgagcaccgcattggaggcatcaagctgcggcatcagcagtggagcctggtcatggaaagcgtggtgccctcggaccgcggcaactacacctgcgtcgtggagaacaagtttggcagcatccggcagacgtacacgctggacgtgctggagcgctccccgcaccggcccatcctgcaggctgggctgcctgctaaccagacagcggtgctgggcagcgacgtggagttccactgcaaggtgtacagtgacgcacagccccacatccagtggctcaagcacgtggaggtgaatggcagcaaggtgggcccggacggcacaccctacgttaccgtgctcaagacggcgggcgctaacaccaccgacaaggagctagaggttctctccttgcacaacgtcacctttgaggacgccggggagtacacctgcctggcgggcaattctattgggttttctcatcactctgcgtggctggtggtgctgccagtgtccctggagtccaacgcgtccatgagctccaacacatga

SEQ ID NO: 38 - protein, 216 aa, Homo sapiens
MRSGCVVVHVWILAGLWLAVAGRPLAFSDAGPHVHYGWGDPIRLRHLYTSGPHGLSSCFLRIRADGVVDCARGQSAHSLLEIKAVALRTVAIKGVHSVRYLCMGADGKMQGLLQYSEEDCAFEEEIRPDGYNVYRSEKHRLPVSLSSAKQRQLYKNRGFLPLSHFLPMLPMVPEEPEDLRGHLESDMFSSPLETDSMDPFGLVTGLEAVRSPSFEK

SEQ ID NO: 39 - protein, 209 aa, Homo sapiens
MDSDETGFEHSGLWVSVLAGLLLGACQAHPIPDSSPLLQFGGQVRQRYLYTDDAQQTEAHLEIREDGTVGGAADQSPESLLQLKALKPGVIQILGVKTSRFLCQRPDGALYGSLHFDPEACSFRELLLEDGYNVYQSEAHGLPLHLPGNKSPHRDPAPRGPARFLPLPGLPPALPEPPGILAPQPPDVGSSDPLSMVGPSQGRSPSYAS